European Patent Application EP 4 541 889 A1, published April 23, 2025. Title: Single-stranded oligonucleotide labeled with fluorescent and quencher. Applicant: TOPPAN PRINTING CO., LTD. The sequence listing filed with the application follows.

SEQUENCE LISTING (2 sequences)

SEQ ID NO: 1 - DNA, 34 bp, synthetic construct
  source 1..34: mol_type = other DNA
  misc_feature 1: note = Modified with ATTO488
  misc_feature 4: note = Modified with BHQ-1
tcttagccggttttccggctaagacctcggcgcg

SEQ ID NO: 2 - DNA, 34 bp, synthetic construct
  source 1..34: mol_type = other DNA
  misc_feature 1: note = Modified with ATTO488
  misc_feature 4: note = Modified with BHQ-1
tcttagccggttttccggctgagacctcggcgcg